European Patent Application EP 4 567 126 A1, published June 11, 2025. Title: 評価方法、複合体及びキット. Applicant: 凸版印刷株式会社. Application WO. The sequence listing filed with the application follows.

SEQUENCE LISTING (4 sequences)

SEQ ID NO: 1 - DNA, 51 bp, synthetic construct
  source 1..51: mol_type = other DNA
tttgtcactgttcctccttttgttttcctttctgtgagcaatttcacccaa

SEQ ID NO: 2 - DNA, 22 bp, synthetic construct
  source 1..22: mol_type = other DNA
gcatggttccaatttgggtgat

SEQ ID NO: 3 - DNA, 28 bp, synthetic construct
  source 1..28: mol_type = other DNA
cgcgccgaggaattgctcacagaaagga

SEQ ID NO: 4 - DNA, 35 bp, synthetic construct
  source 1..35: mol_type = other DNA
ttcttagccggttttccggctgagacctcggcgcg